European Patent Specification EP 4 172 301 B1, published July 24, 2024. Title: Low diacetyl yeast. Applicant: Carlsberg A/S. The sequence listing filed with the application follows.

SEQUENCE LISTING (74 sequences)

SEQ ID NO: 1 - DNA, 19 bp, Artificial sequence
  ILV2 forward primer
  primer_bind (1)..(19): ILV2 forward primer
gccaacgacacaggaagac

SEQ ID NO: 2 - DNA, 20 bp, Artificial sequence
  ILV2 reverse primer
  primer_bind (1)..(20): ILV2 reverse primer
gtacctaaaccacctgatgt

SEQ ID NO: 3 - DNA, 15 bp, Artificial sequence
  ILV2 S. cerevisiae probe
  misc_feature (1)..(15): ILV2 S. cerevisiae probe
tgggctgctcaacac

SEQ ID NO: 4 - DNA, 18 bp, Artificial sequence
  ILV2 S. eubayanus probe
  misc_feature (1)..(18): ILV2 S. eubayanus probe
acgtacggaatgtggatt

SEQ ID NO: 5 - protein, 687 aa, Saccharomyces cerevisiae
MIRQSTLKNFAIKRCFQHIAYRNTPAMRSVALAQRFYSSSSRYYSASPLPASKRPEPAPSFNVDPLEQPAEPSKLAKKLRAEPDMDTSFVGLTGGQIFNEMMSRQNVDTVFGYPGGAILPVYDAIHNSDKFNFVLPKHEQGAGHMAEGYARASGKPGVVLVTSGPGATNVVTPMADAFADGIPMVVFTGQVPTSAIGTDAFQEADVVGISRSCTKWNVMVKSVEELPLRINEAFEIATSGRPGPVLVDLPKDVTAAILRNPIPTKTTLPSNALNQLTSRAQDEFVMQSINKAADLINLAKKPVLYVGAGILNHADGPRLLKELSDRAQIPVTTTLQGLGSFDQEDPKSLDMFGMHGCATANLAVQNADLIIAVGARFDDRVTGNISKFAPEARRAAAEGRGGIIHFEVSPKNINKVVQTQIAVEGDATTNLGKMMSKIFPVKERSEWFAQINKWKKEYPYAYMEETPGSKIKPQTVIKKLSKVANDTGRHVIVTTGVGQHQMWAAQHWTWRNPHTFITSGGLGTMGYGLPAAIGAQVAKPESLVIDIDGDASFNMTLTELSSAVQAGTPVKILILNNEEQGMVTQWQSLFYEHRYSHTHQLNPDFIKLAEAMGLKGLRVKKQEELDAKLKEFVSTKGPVLLEVEVDKKVPVLPMVAGGSGLDEFINFDPEVERQQTELRHKRTGGKH

SEQ ID NO: 6 - protein, 309 aa, Saccharomyces cerevisiae
MLRSLLQSGHRRVVASSCATMVRCSSSSTSALAYKQMHRHATRPPLPTLDTPSWNANSAVSSIIYETPAPSRQPRKQHVLNCLVQNEPGVLSRVSGTLAARGFNIDSLVVCNTEVKDLSRMTIVLQGQDGVIEQARRQIEDLVPVYAVLDYTNSEIVKRELVMARISLLGTEYFEDLLLHHHTSTNAGAADSQELVAEIREKQFHPANLPASEVLRLKHEHLNDITNLTNNFGGRVVDISETSCIVELSAKPTRISAFLKLVEPFGVLECARSGMMALPRTPLKTSTEEAADEDEKISEIVDISQLPPG

SEQ ID NO: 7 - protein, 309 aa, Saccharomyces eubayanus
MLRSLLQSGHRRVAASSCATMVRCSSSSTSALAYKQMHRHAARPPLPTLDTPSWNANSAVSSIIYETPAPSRQPRKQHVLNCLVQNEPGVLSRISGTLAARGFNIDSLVVCNTEVKDLSRMTIVLQGQDGVIEQARRQIEDLVPVYAVLDYTNSEIIKRELVMARISLLGTEYFEDLLLHHHTSTSSGGADANELVAEIREKQFHPANLPASEILRLKHEHLNDVTNLTNNFGGRVVDISETSCIVELSAKPTRISAFLKLVEPFGVLECARSGMMALPRTPLKTSIEEAADEDEKINEIVDISQLPPG

SEQ ID NO: 8 - protein, 395 aa, Saccharomyces Cerevisiae
MLRTQAARLICNSRVITAKRTFALATRAAAYSRPAARFVKPMITTRGLKQINFGGTVETVYERADWPREKLLDYFKNDTFALIGYGSQGYGQGLNLRDNGLNVIIGVRKDGASWKAAIEDGWVPGKNLFTVEDAIKRGCYVMNLLSDAAQSETWPAIKPLLTKGKTLYFSHGFSPVFKDLTHVEPPKDLDVILVAPKGSGRTVRSLFKEGRGINSSYAVWNDVTGKAHEKAQALAVAIGSGYVYQTTFEREVNSDLYGERGCLMGGIHGMFLAQYDVLRENGHSPSEAFNETVEEATQSLYPLIGKYGMDYMYDACSTTARRGALDWYPIFKNALKPVFQDLYESTKNGTETKRSLEFNSQPDYREKLEKELDTIRNMEIWKVGKEVRKLRPENQ

SEQ ID NO: 9 - protein, 395 aa, Saccharomyces eubayanus
MLRTQAARLICNSRVVTAKRTFALATRAAAYSRPAARFVKPMVATRGLKQINFGGTVETVYERADWPREKLLNYFKDDTFALIGYGSQGYGQGLNLRDNGLNVIIGVRKDGASWKAAIEDGWVPGQNLFSVEDAIKKGNYVMNLLSDAAQSETWPTIKPLLTKGKTLYFSHGFSPVFKDLTHVEPPKDLDVILVAPKGSGRTVRSLFKEGRGINSSYAVWNDVTGKAHEKAQALAVAIGSGYVYQTTFEREVNSDLYGERGCLMGGIHGMFLAQYDVLRENGHSPSEAFNETVEEATQSLYPLIGKYGMDYMYDACSTTARRGALDWYPIFKNALKPVFQDLYESTKNGTETKRSLEFNSQPDYREKLEKELVTIRNMEIWKVGKEVRKLRPENK

SEQ ID NO: 10 - protein, 585 aa, Saccharomyces cerevisiae
MGLLTKVATSRQFSTTRCVAKKLNKYSYIITEPKGQGASQAMLYATGFKKEDFKKPQVGVGSCWWSGNPCNMHLLDLNNRCSQSIEKAGLKAMQFNTIGVSDGISMGTKGMRYSLQSREIIADSFETIMMAQHYDANIAIPSCDKNMPGVMMAMGRHNRPSIMVYGGTILPGHPTCGSSKISKNIDIVSAFQSYGEYISKQFTEEEREDVVEHACPGPGSCGGMYTANTMASAAEVLGLTIPNSSSFPAVSKEKLAECDNIGEYIKKTMELGILPRDILTKEAFENAITYVVATGGSTNAVLHLVAVAHSAGVKLSPDDFQRISDTTPLIGDFKPSGKYVMADLINVGGTQSVIKYLYENNMLHGNTMTVTGDTLAERAKKAPSLPEGQEIIKPLSHPIKANGHLQILYGSLAPGGAVGKITGKEGTYFKGRARVFEEEGAFIEALERGEIKKGEKTVVVIRYEGPRGAPGMPEMLKPSSALMGYGLGKDVALLTDGRFSGGSHGFLIGHIVPEAAEGGPIGLVRDGDEIIIDADNNKIDLLVSDKEMAQRKQSWVAPPPRYTRGTLSKYAKLVSNASNGCVLDA

SEQ ID NO: 11 - protein, 585 aa, Saccharomyces eubayanus
MGLLTKVATSRQFSTTRSVAKKLNKYSYIITEPKGQGASQAMLYATGFKKDDFQKPQVGVGSCWWSGNPCNMHLLDLNNRCSQSIEKAGLKAMQFNTIGVSDGISMGTKGMRYSLQSREIIADSFETIMMAQHYDANIAIPSCDKNMPGVMMAMGRHNRPSIMVYGGTILPGHPTCGSSKISKNIDIVSAFQSYGEYISKQFTEEEREDVVEHACPGPGSCGGMYTANTMASAAEVLGLTIPNSSSFPAVSKQKLAECDNIGEYIKTTMELGILPRDILTKEAFENAITYVVATGGSTNAVLHLVAVAHSAGVKLSPDDFQRISNTTPLIGDFKPSGKYVMADLINVGGTQSVIKYLYENNMLHGNTMTVTGDTLAERAKKAPSLPEGQEIIKPLSHPIKTSGHLQILYGSLAPGGAVGKITGKEGTYFKGKARVYEEEGAFIEALEKGEIKKGEKTVVIIRYEGPRGAPGMPEMLKPSSALMGYGLGKDVALLTDGRFSGGSHGFLIGHIVPEAAEGGPIGLVKDGDEIIIDADNNKIDLLISEQEMSQRKQNWVAPPPRYTRGTLSKYAKLVSNASSGCVLDA

SEQ ID NO: 12 - protein, 585 aa, Saccharomyces cerevisiae; identical to SEQ ID NO: 10

SEQ ID NO: 13 - protein, 585 aa, Saccharomyces eubayanus; identical to SEQ ID NO: 11

SEQ ID NO: 14 - protein, 393 aa, Saccharomyces cerevisiae
MLQRHSLKLGKFSIRTLATGAPLDASKLKITRNPNPSKPRPNEELVFGQTFTDHMLTIPWSAKEGWGTPHIKPYGNLSLDPSACVFHYAFELFEGLKAYRTPQNTITMFRPDKNMARMNKSAARICLPTFESEELIKLTGKLIEQDKHLVPQGNGYSLYIRPTMIGTSKGLGVGTPSEALLYVITSPVGPYYKTGFKAVRLEATDYATRAWPGGVGDKKLGANYAPCILPQLQAAKRGYQQNLWLFGPEKNITEVGTMNVFFVFLNKVTGKKELVTAPLDGTILEGVTRDSVLTLARDKLDPQEWDINERYYTITEVATRAKQGELLEAFGSGTAAVVSPIKEIGWNNEDIHVPLLPGEQCGALTKQVAQWIADIQYGRVNYGNWSKTVADLN

SEQ ID NO: 15 - protein, 393 aa, Saccharomyces cerevisiae; identical to SEQ ID NO: 14

SEQ ID NO: 16 - protein, 393 aa, Saccharomyces eubayanus
MLQRNSLKWGKFSIRTLATGAPLDASKLKITRNPNPSKPRPNDELVFGQTFTDHMLTIPWTAKEGWGVPHIKPYANLSLDPSSCVFHYAFELFEGLKAYRTPQNTITMFRSDKNMVRMNKSAARICLPTFDSEELIKLTGKLIEQDKHLVPEGNGYSLYIRPTMIGTSKGLGVGTPSEALLYVITSPVGPYYKTGFKAVRLEATDYATRAWPGGVGDKKLGANYAPCILPQLQAAKRGYQQNLWLFGPEKNITEVGTMNVFFVFLNKVTGKKELVTAPLDGTILEGVTRDSVLSLAREKLDPQEWDINERYYTITEVATRAQQGELLEAFGSGTAAVVSPIKEIGWKDQDINVPLLPGEQSGALTKQVAQWIADIQYGRTKHGNWSRTVADLN

SEQ ID NO: 17 - protein, 376 aa, Saccharomyces cerevisiae
MTLAPLDASKVKITTTQHASKPKPNSELVFGKSFTDHMLTVEWTAEKGWGTPEIKPYQNLSLDPSAVVFHYAFELFEGMKAYRTVDNKITMFRPDMNMKRMNKSAQRICLPTFDPEELITLIGKLIQQDKYLVPEGKGYSLYIRPTLIGTTAGLGVSTPDRALLYVICCPVGPYYKTGFKAVRLEATDYATRAWPGGCGDKKLGANYAPCVLPQLQAASRGYQQNLWLFGPNNNITEVGTMNAFFVFKDSKTGKKELVTAPLDGTILEGVTRDSILNLAKERLEPSEWTISERYFTIGEVTERSKNGELLEAFGSGTAAIVSPIKEIGWKGEQINIPLLPGEQTGPLAKEVAQWINGIQYGETEHGNWSRVVTDLN

SEQ ID NO: 18 - protein, 376 aa, Saccharomyces eubayanus
MTLAPLDASKVKITTTQHASKPKPNSELVFGKSFTDHMLTAEWTAEKGWGTPEIKPYQNLSLDPSAVVFHYAFELFEGMKAYRTVDNKITMFRPDMNMKRMNKSAQRICLPTFDPEELITLIGKLIQQDKYLVPEGKGYSLYIRPTLIGTTAGLGVSTPDRALLYVICCPVGPYYKTGFKAVRLEATDYATRAWPGGCGDKKLGANYAPCVLPQLQAASRGYQQNLWLFGPNNNITEVGTMNAFFVFKDSKTGKKELVTAPLDGTILEGVTRDSILNLAKERLEPSEWTISERYFTIGEVTERSKNGELLEAFGSGTAVIVSPIKEIGWKGEQINIPLLPGEQTGPLAKEVAQWINGIQYGETEHGNWSRVVTDLN

SEQ ID NO: 19 - protein, 374 aa, Saccharomyces eubayanus
LAPLDASKVKITTTEHPSEPKPNDQLVFGRSFTDHMLTAEWTAANGWDVPEIKPYQNLSLDPSAYVFHYAFELFEGMKAYRTVDNKITMFRPDMNMKRMNKSARRICLPAFDSEELIALIAKLIQQDKRLIPEGKGYSLYIRPTMIGTTAGLGVSTPDRALLYVICSPVGPYYKTGFKAVRLEATDYATRAWPGGCGDKKLGANYAPCVLPQLQAASRGYQQNLWLFGPENNITEVGTMNAFFVFKNTETGKKELVTAPLDGTILEGVTRDSILTLAKERLDLNEWTISERYCTIGEVSERSKKGELVEAFGSGTAAIVSPIKEIGWKGEPINIPLLPGEQTGPLTKEVAQWINQIQYGEVEHGNWSRVITDLN

SEQ ID NO: 20 - protein, 687 aa, Saccharomyces cerevisiae
MIRQSTLKNFAIKRCFQHIAYRNTPAMRSVALAQRFYSSSSRYYSASPLPASKRPEPAPSFNVDPLEQPAEPSKLAKKLRAEPDMDTSFVGLTGGQIFNEMMSRQNVDTVFGYPGGAILPVYDAIHNSDKFNFVLPKHEQGAGHMAEGYARASGKPGVVLVTSGPGATNVVTPMADAFADGIPMVVFTGQVSTSAIGTDAFQEADVVGISRSCTKWNVMVKSVEELPLRINEAFEIATSGRPGPVLVDLPKDVTAAILRNPIPTKTTLPSNALNQLTSRAQDEFVMQSINKAADLINLAKKPVLYVGAGILNHADGPRLLKELSDRAQIPVTTTLQGLGSFDQEDPKSLDMFGMHGCATANLAVQNADLIIAVGARFDDRVTGNISKFAPEARRAAAEGRGGIIHFEVSPKNINKVVQTQIAVEGDATTNLGKMMSKIFPVKERSEWFAQINKWKKEYPYAYMEETPGSKIKPQTVIKKLSKVANDTGRHVIVTTGVGQHQMWAAQHWTWRNPHTFITSGGLGTMGYGLPAAIGAQVAKPESLVIDIDGDASFNMTLTELSSAVQAGTPVKILILNNEEQGMVTQWQSLFYEHRYSHTHQLNPDFIKLAEAMGLKGLRVKKQEELDAKLKEFVSTKGPVLLEVEVDKKVPVLPMVAGGSGLDEFINFDPEVERQQTELRHKRTGGKH

SEQ ID NO: 21 - protein, 309 aa, Saccharomyces cerevisiae; identical to SEQ ID NO: 6

SEQ ID NO: 22 - protein, 309 aa, Saccharomyces eubayanus; identical to SEQ ID NO: 7

SEQ ID NO: 23 - protein, 395 aa, Saccharomyces cerevisiae; identical to SEQ ID NO: 8

SEQ ID NO: 24 - protein, 395 aa, Saccharomyces eubayanus; identical to SEQ ID NO: 9

SEQ ID NO: 25 - protein, 585 aa, Saccharomyces cerevisiae; identical to SEQ ID NO: 10

SEQ ID NO: 26 - protein, 585 aa, Saccharomyces eubayanus; identical to SEQ ID NO: 11

SEQ ID NO: 27 - protein, 585 aa, Saccharomyces eubayanus; identical to SEQ ID NO: 11

SEQ ID NO: 28 - protein, 393 aa, Saccharomyces cerevisiae; identical to SEQ ID NO: 14

SEQ ID NO: 29 - protein, 393 aa, Saccharomyces eubayanus; identical to SEQ ID NO: 16

SEQ ID NO: 30 - protein, 376 aa, Saccharomyces cerevisiae; identical to SEQ ID NO: 18

SEQ ID NO: 31 - protein, 374 aa, Saccharomyces eubayanus; identical to SEQ ID NO: 19

SEQ ID NO: 32 - protein, 687 aa, Saccharomyces cerevisiae [sequence omitted]

SEQ ID NO: 33 - protein, 309 aa, Saccharomyces cerevisiae [sequence omitted]

SEQ ID NO: 34 - protein, 395 aa, Saccharomyces cerevisiae
MLRTQAARLICNSRVITAKRTFALATRAAAYSRPAARFVKPMITTRGLKQINFGGTVETVYERADWPREKLLDYFKNDTFALIGYGSQGYGQGLNLRDNGLNVIIGVRKDGASWKAAIEDGWVPGKNLFTVEDAIKRGSYVMNLLSDAAQSETWPAIKPLLTKGKTLYFSHGFSPVFKDLTHVEPPKDLDVILVAPKGSGRTVRSLFKEGRGINSSYAVWNDVTGKAHEKAQALAVAIGSGYVYQTTFEREVNSDLYGERGCLMGGIHGMFLAQYDVLRENGHSPSEAFNETVEEATQSLYPLIGKYGMDYMYDACSTTARRGALDWYPIFKNALKPVFQDLYESTKNGTETKRSLEFNSQPDYREKLEKELDTIRNMEIWKVGKEVRKLRPENQ

SEQ ID NO: 35 - protein, 585 aa, Saccharomyces cerevisiae; identical to SEQ ID NO: 10

SEQ ID NO: 36 - protein, 393 aa, Saccharomyces cerevisiae; identical to SEQ ID NO: 14

SEQ ID NO: 37 - protein, 376 aa, Saccharomyces cerevisiae; identical to SEQ ID NO: 17

SEQ ID NO: 38 - protein, 687 aa, Saccharomyces eubayanus
MIRQSTLKNFAIKRCFQQMAYRNTPAMRSVALAQRFYSSSSRYYSASPLPASNRPEPAPSFNVEPVAQVPEPSKLAKRLRTEPDMDTSFVGLTGGQIFNEMMSRHNVDTVFGYPGGAILPVYDAIHNSDKFTFVLPRHEQGAGHMAEGYARASGKPGVVLVTSGPGATNVITPMADAFADGIPMVVFTGQVPTSAIGTDAFQEADVVGISRSCTKWNVMVKTVEELPLRINEAFEIATSGRPGPVLVDLPKDVTAAILRNPIPTKTTLPSNALNQLTSRTQDEFVLQNINRAADLINLAKKPVLYVGAGILNHADGPRLLKELSDRAQIPVTTTLQGLGAFDQDDPKSLDMLGMHGCATANLAVQNADLLIAVGARFDDRVTLNIAKFAPEARRAAAEGRGGIIHFEVSPKNINKVVETQIAVEGDATGNLDKMMPKIFPVKERSEWFGQINEWKKKYPYAYMMETPGSKIKPQTVITKLSKIANDTGRHVIVTTGVGQHQMWAAQHWTWKTPRTFITSGGLGTMGYGLPAAIGAQVAKPDSLVIDIDGDASFNMTLTELSSAVQAGTPVKILVLNNEEQGMVTQWQSLFYENRYSHTHQLNPDFIKLADAMGLKGLRVKKQEELDAKLKEFVSTKGPVLLEVEVDKKVPVLPMVPAGKGLDEFIYFDPEVERQQNELRHKRTNGKH

SEQ ID NO: 39 - protein, 309 aa, Saccharomyces eubayanus; identical to SEQ ID NO: 7

SEQ ID NO: 40 - protein, 395 aa, Saccharomyces eubayanus; identical to SEQ ID NO: 9

SEQ ID NO: 41 - protein, 585 aa, Saccharomyces eubayanus; identical to SEQ ID NO: 11

SEQ ID NO: 42 - protein, 393 aa, Saccharomyces eubayanus
MLQRNSLKLGKFSIRTLATGAPLDASKLKITRNPNPSKPRPNDELVFGQTFTDHMLTIPWTAKEGWGVPHIKPYANLSLDPSSCVFHYAFELFEGLKAYRTPQNTITMFRSDKNMVRMNKSAARICLPTFDSEELIKLTGKLIEQDKHLVPEGNGYSLYIRPTMIGTSKGLGVGTPSEALLYVITSPVGPYYKTGFKAVRLEATDYATRAWPGGVGDKKLGANYAPCILPQLQAAKRGYQQNLWLFGPEKNITEVGTMNVFFVFLNKVTGKKELVTAPLDGTILEGVTRDSVLTLAREKLDPQEWDINERYYTITEVATRAQQGELLEAFGSGTAAVVSPIKEIGWKDQDINVPLLPGEQSGALTKQVAQWIADIQYGRTKHGNWSRTVADLN

SEQ ID NO: 43 - protein, 376 aa, Saccharomyces eubayanus
MTLAPLDASKVKITTTEHPSEPKPNDQLVFGRSFTDHMLTVEWTAANGWDVPEIKPYQNLSLDPSAYVFHYAFELFEGMKAYRTVDNKITMFRPDMNMKRMNKSAQRICLPAFDSEELIALIAKLIQQDKRLIPEGKGYSLYIRPTMIGTTAGLGVSTPDRALLYVICSPVGPYYKTGFKAVRLEATDYATRAWPGGCGDKKLGANYAPCVLPQLQAASRGYQQNLWLFGPENNITEVGTMNAFFVFKDTETGKKELVTAPLDGTILEGVTRDSILTLAKERLDLDEWTISERYCTIGEVSERSKKGELVEAFGSGTAAIVSPIKEIGWKGEPINIPLLPGEQTGPLTKEVAQWINQIQYGEVEHGNWSRVITDLN

SEQ ID NO: 44 - DNA, 71 bp, Artificial
  Primer
  misc_feature (1)..(71): CPA43
caacaaatggcataccgtaacacacctgctatgagatcagtcgccctcgcggctagctcgagcccacacac

SEQ ID NO: 45 - DNA, 72 bp, Artificial
  Primer
  misc_feature (1)..(72): CPA44
ggatcaaagtatatgaactcatctagacccttgcctgctggaaccattgggatccccgggaattcagcttgc

SEQ ID NO: 46 - DNA, 24 bp, Artificial
  Primer
  misc_feature (1)..(24): CPA49
cggtaccggcttggaatagccatg

SEQ ID NO: 47 - DNA, 25 bp, Artificial
  Primer
  misc_feature (1)..(25): CPA50
gaacaccgatcttagattgtactga

SEQ ID NO: 48 - DNA, 30 bp, Artificial
  Primer
  misc_feature (1)..(30): CPA51
gcaggtgtgttacggtatgccatttgttgg

SEQ ID NO: 49 - DNA, 34 bp, Artificial
  Primer
  misc_feature (1)..(34): CPA52
gggtctagatgagttcatatactttgatccagag

SEQ ID NO: 50 - DNA, 2213 bp, Artificial
  Knockout cassette
  misc_feature (1)..(2213): ILV2 (se) knockout cassette
cggtaccggcttggaatagccatgaatctcggcgcggaaatatcagcgccctccgccgaaatgttgggaaatcgtctttttctttctttttttctgaatctttcatctattcgatagcgatgattcatttcttctgaaaaaaaaaaaatagaaatttttattaacatgtaattctcttatccgtttaatatatatgctatcgtttattctcttatcgaattttcatttctattcccttccgccatccctaattcaaagtacagatccacgttactattgtaaattgcttgtttttttgccttcactgtttttaaattatcagccacagttactttagtcatctgaagtgaagattgcatacttttactgattacaataaattgcattaacatagtctatacgcataggagaaaacacacaatagaaatccactcgccaaatgatcagacagtccacactcaagaacttcgctattaagcgttgcttccaacaaatggcataccgtaacacacctgctatgagatcagtcgccctcgcggctagctcgagcccacacaccatagcttcaaaatgtttctactccttttttactcttccagattttctcggactccgcgcatcgccgtaccacttcaaaacacccaagcacagcatactaaattttccctctttcttcctctagggtgtcgttaattacccgtactaaaggtttggaaaagaaaaaagagaccgcctcgtttctttttcttcgtcgaaaaaggcaataaaaatttttatcacgtttctttttcttgaaatttttttttttagtttttttctctttcagtgacctccattgatatttaagttaataaacggtcttcaatttctcaagtttcagtttcatttttcttgttctattacaactttttttacttcttgttcattagaaagaaagcatagcaatctaatctaaggggcggtgttgacaattaatcatcggcatagtatatcggcatagtataatacgacaaggtgaggaactaaaccatggctaaattgacatctgctgttccagttttgactgctagagatgttgctggtgctgttgaattttggactgatagattgggtttctccagagatttcgttgaagatgatttcgctggtgttgttagagatgatgttaccttgtttatctccgccgttcaagatcaagttgttccagataatactttggcttgggtttgggttagaggtttggatgaattatatgccgaatggtccgaagttgtttctaccaattttagagatgcttctggtccagctatgaccgaaattggtgaacaaccatggggtagagaatttgctttgagagatccagctggtaactgtgttcattttgttgctgaagaacaggactaacacgtccgacggcggcccacgggtcccaggcctcggagatccgtcccccttttcctttgtcgatatcatgtaattagttatgtcacgcttacattcacgccctccccccacatccgctctaaccgaaaaggaaggagttagacaacctgaagtctaggtccctatttatttttttatagttatgttagtattaagaacgttatttatatttcaaatttttcttttttttctgtacagacgcgtgtacgcatgtaacattatactgaaaaccttgcttgagaaggttttgggacgctcgaaggctttaatttgcaagctgaattcccggggatcccaatggttccagcaggcaagggtctagatgagttcatatactttgatccagaggttgaaagacaacaaaatgaattacgtcacaagcgtaccaatggtaagcattgaagtctgaaacacattctccattaaaaatttagacttaattattatttaaccatgcttatatagtacatcctgtcctacgacaaacacgtatacttttttaataaatttctttttttaaactattcacaactagcctttaaccatgatgagtagcaagtcacacgtccgagtaggcattagcacatcattagtgaatacttcacgcaatgacatgaagcttcttttcctcgtctgacacgatttcttctttagtaaattgtcaaaaatatttccgaaaaggggccgctaaaaaatgcattctctgttaatattgatctactgctgtaaataaatgataaaactttcagtacaatctaagatcggtgttc

SEQ ID NO: 51 - DNA, 29 bp, Artificial
  Primer
  misc_feature (1)..(29): CPA70
gttctgacctgctgcaacctccaatactc

SEQ ID NO: 52 - DNA, 34 bp, Artificial
  Primer
  misc_feature (1)..(34): CPA71
gcctgtccataatatcattgatatctatagagtg

SEQ ID NO: 53 - DNA, 27 bp, Artificial
  Primer
  misc_feature (1)..(27): CPA91
gcccgggctcgaatcgacagcagtata

SEQ ID NO: 54 - DNA, 34 bp, Artificial
  Primer
  misc_feature (1)..(34): CPA96
gatattatggacaggcgctagctcgagcccacac

SEQ ID NO: 55 - DNA, 31 bp, Artificial
  Primer
  misc_feature (1)..(31): CPA111
ggcaagggacaccatacatcacctaatgctg

SEQ ID NO: 56 - DNA, 35 bp, Artificial
  Primer
  misc_feature (1)..(35): CPA112
gttgcagcaggtcagaacttcttggaaataggagc

SEQ ID NO: 57 - DNA, 30 bp, Artificial
  Primer
  misc_feature (1)..(30): CPA113
cgattcgagcccgggcgctttggcatccac

SEQ ID NO: 58 - DNA, 35 bp, Artificial
  Primer
  misc_feature (1)..(35): CPA114
gatatgcggtattcgtttacattcctgatatattc

SEQ ID NO: 59 - DNA, 35 bp, Artificial
  Primer
  misc_feature (1)..(35): CPA128
tattatggacaggcgctagctcgagcccacacacc

SEQ ID NO: 60 - DNA, 35 bp, Artificial
  Primer
  misc_feature (1)..(35): CPA129
tcgagctagcgcctgtccataatatcattgatatc

SEQ ID NO: 61 - DNA, 5307 bp, Artificial
  Integration cassette
  misc_feature (1)..(5307): ILV3 (se) NTC integration cassette
ggcaagggacaccatacatcacctaatgctgttaattataaccaacttgacaacgattgcacaagaaaagagtatacctgtgaagacagccaaaacgcttaacatgttatgacataaattgcagacaagaaattggatgtattttacagactttgcattcctgtctgaaagcctttttacataaaaatggtttcattagtagcacttcgtatcgttttcaaataatgatgagatgctccaaaaggaaagttggcacagaaaaaatgacgcgcctttcctgtttaccgttaaacttctcagaaaaagtatactcgacccatttttaagattggtgatggatagaatttcatttaacataatgctgcaaatatagattgatttcaatctacggagtccaacgcattgaacagcttcaattgaatagatatgctcctatttccaagaagttctgacctgctgcaacctccaatactcatacacatctctatatattcaatctttaatctttactgtcatcttccacatatcattcctcacgagcgggcacctactatttttccccctctgtttaaggtgaaaagggccccaatgctaccagcttttacctccacacgactctccacacagcagcaaccacacagcaatgccatccgacgcagcagccagcaccggcctgcccacgccgtggactgtcaggtacagcaagtccaagaaaagagagtacttcttcaacccggacacgaagcactcgcagtgggaggagcccgagggtacggataaggaacagctgcacgagtatctgaaagaccacccaatgcgtgtaaggtgtctgcacatcctcatcaagcaccaggactcgagaagacctgcttcgcaccggtccgagaacatcaccatatccaagcaagaggccacggacgagctaaagaccctggtcacgaggctggacgacgcttccaagaccaactccttcgaggcgctggctaaggagaggtccgactgctcttcgtacaagaggggcggcgacctgggctggttcggcaggggcgagatgcagcccagtttcgaggacgccgccttcaagctcaaggtcggagaagtgagcgacattgtcgagtcgggcagcggtgtccatttaatcaagcgtgtgggttagtcgtccgccctaatccctactctccaaatcacgttgttgcttcacctcacactcgaacgcacgaaaaaattctaaaatactagaggcattactaacgctgcctttttgttacgagcggaaccggacatgaaaaaaaaaattttcttttaacttttttcaccagatgactcaataaattattagtacattatataatataacaaaagaagagactggtctttttagcgtgtacacacatactctctagttataacgtttcttgttttctcatttgcaaatacaaccaagaagtatcagcagagatgggcttgttaacgaaagtagccacgtcgagacaattctctacaacgagatccgttgccaagaaactaaacaagtattcctacatcatcactgaaccaaagggccaaggtgcctcccaggccatgctttacgctaccgggttcaagaaggatgacttccaaaagcctcaggttggtgtcggttcatgctggtggtctggtaacccatgcaacatgcatctgttggacttgaacaacagatgttcccaatccatcgaaaaggctggcctaaaggccatgcagttcaacaccatcggtgtttctgacggtatctccatgggtaccaagggtatgagatactctttgcaaagtagagagatcattgcggactcgtttgaaaccatcatgatggctcagcattacgatgccaacatcgccatcccatcttgtgacaagaacatgcccggtgtcatgatggccatgggtagacacaatagaccctccatcatggtctacggtggtaccatcttgcccggtcacccaacctgcgggtcctccaagatctccaaaaacatcgacattgtctcagctttccaatcttacggtgagtatatctccaagcagttcactgaagaagagagagaagatgtcgtggaacacgcctgccctggtcctggttcttgtggtggtatgtacaccgccaacacaatggcctctgccgcagaagtcctaggtttaaccattccaaactcctcttccttccccgccgtgtccaagcagaagttggccgagtgtgacaatattggtgaatacatcaagacaacaatggaattgggcattttgccccgtgacatcctcaccaaggaggcctttgaaaatgccattacttacgtcgttgccacaggtgggtccaccaatgctgttttgcatctggttgccgttgctcattccgcgggtgttaagttgtctccagatgatttccaaagaatcagtaacaccacaccattgatcggtgacttcaagccttccggtaaatacgtcatggctgacttgatcaacgtcggtggtacacaatccgtgattaagtacctatacgaaaacaacatgttacatggtaacaccatgactgtcaccggtgacactttggcagaacgtgccaagaaggcaccaagcttgcctgaaggccaagagatcatcaaacctctttcccatccaatcaagaccagcggtcacttacaaatcttatacggttcattggcgccaggtggtgccgtgggtaaaattaccggtaaggaaggtacttacttcaaaggtaaggcccgtgtctacgaagaagaaggtgcctttattgaagctttggaaaagggcgaaatcaagaagggtgaaaaaactgttgttattatcagatacgaaggtccaagaggtgctccaggtatgcctgaaatgctaaagccttcttctgctctaatggggtacggtttaggtaaagatgtcgcattgttgactgatggtagattctccggtggttctcatgggttcttgatcggtcacattgtcccagaagccgctgaaggtggacctattggtcttgtgaaagacggtgacgaaatcattatcgatgctgacaacaacaagattgatttgttgatctccgaacaggaaatgtctcaacgtaagcaaaactgggtcgctcctccacctcgttacacaagaggtactttatccaaatatgctaagttggtttccaacgcttccagcggttgtgtcctagatgcttgatgcattataggcaccaatcgatgaatatatatacagattctcctttcctcattttttctcacccccaatctttttctttatatatataaatatttattatagtccattgaatggataaaacatttatttaaaaaaatcctattttttttacaagtctcagttggtaatgtatccaccattactggccctgttgtgatgcagctaaggccttttgtctcaattttctgcccgcgtatttactgacaaatggtaacaatgcggtatttaatgcaatgagggcaactaaaataccataattcctccccatcttgcctcttgacaagtcaaaaaaaatcactctatagatatcaatgatattatggacaggcgctagctcgagcccacacaccatagcttcaaaatgtttctactccttttttactcttccagattttctcggactccgcgcatcgccgtaccacttcaaaacacccaagcacagcatactaaattttccctctttcttcctctagggtgtcgttaattacccgtactaaaggtttggaaaagaaaaaagagaccgcctcgtttctttttcttcgtcgaaaaaggcaataaaaatttttatcacgtttctttttcttgaaatttttttttttagtttttttctctttcagtgacctccattgatatttaagttaataaacggtcttcaatttctcaagtttcagtttcatttttcttgttctattacaactttttttacttcttgttcattagaaagaaagcatagcaatctaatctaaggggcggtgttgacaattaatcatcggcatagtatatcggcatagtataatacgacaaggtgaggaactaaaccatgggtactactttggatgataccgcttatagatacagaacttctgttccaggtgatgctgaagctattgaagctttggatggttctttcactactgacactgttttcagagttactgctactggtgatggtttcactttgagagaagttccagttgatccaccattgactaaggtttttccagatgatgaatccgatgacgaatctgatgatggtgaagatggtgatccagattctagaacttttgttgcttatggtgatgacggtgatttggctggttttgttgttgtttcttactctggttggaatagaagattgaccgtcgaagatattgaagttgctccagaacatagaggtcatggtgttggtagagctttgatgggtttagctactgaatttgctagagaacgtggtgctggtcatttgtggttggaagttactaatgttaacgctccagctattcatgcctatagaagaatgggttttaccttgtgtggtttggatactgcattatacgatggtactgcttcagatggtgaacaagccttgtatatgtctatgccatgtccatgatcagtactgacaataaaaagattcttgttttcaagaacttgtcatttgtatagtttttttatattgtagttgttctattttaatcaaatgttagcgtgatttatattttttttcgcctcgacatcatctgcccagatgcgaagttaagtgcgcagaaagtaatatcatgcgtcaatcgtatgtgaatgctggtcgctatactgctgtcgattcgagcccgggcgctttggcatccacgctgacacttttcctcgttgggaaggaataaaaagcaagtaacactttttctgagcattttattacgttattcaactactaatagagttgatttgttacttgctaaaatctttttatatttcttttagccccgacagaacttgttgcaaatgaatacaaaccgtgaacttcccgatatcattctaattgaacccagatatttacacatgtacttcttactcattttcaatgtcagcttaaatatcgtctaaaacaatattttactagatacgcagttcaatcttcgcgcatattttcgcgaaagtccaaattgcgtacgtggttttatgtcaaagtgaccgccgttgtagcgtactttttcctataagacaagctcgtgatatcaggaatatatcaggaatgtaaacgaataccgcatatct

SEQ ID NO: 62 - DNA, 25 bp, Artificial
  Primer
  misc_feature (1)..(25): CPA74
gtagtaagtgataagcgaatttggc

SEQ ID NO: 63 - DNA, 31 bp, Artificial
  Primer
  misc_feature (1)..(31): CPA75
gcgtcacagcaaccagtagctcagccaaaac

SEQ ID NO: 64 - DNA, 43 bp, Artificial
  Primer
  misc_feature (1)..(43): CPA86
cttttgctcacatgtgtttgtagtaagtgataagcgaatttgg

SEQ ID NO: 65 - DNA, 35 bp, Artificial
  Primer
  misc_feature (1)..(35): CPA87
ctcacttggccagtttgcgtcacagcaaccagtag

SEQ ID NO: 66 - DNA, 2595 bp, Artificial
  Expression cassette
  misc_feature (1)..(2595): ILV5 (sc) expression cassette
cttttgctcacatgtgtttgtagtaagtgataagcgaatttggctaagaacgttgtaagtgaacaagggacctcttttgcctttcaaaaaaggattaaatggagttaatcattgagatttagttttcgttagattctgtatccctaaataactcccttacccgacgggaaggcacaaaagacttgaataatagcaaacggccagtagccaagaccaaataatactagagttaactgatggtcttaaacaggcattacgtggtgaactccaagaccaatatacaaaatatcgataagttattcttgcccaccaatttaaggagcctacatcaggacagtagtaccattcctcagagaagaggtatacataacaagaaaatcgcgtgaacaccttatataacttagcccgttattgagctaaaaaaccttgcaaaatttcctatgaataagaatacttcagacgtgataaaaatttactttctaactcttctcacgctgcccctatctgttcttccgctctaccgtgagaaataaagcatcgagtacggcagttcgctgtcactgaactaaaacaataaggctagttcgaatgatgaacttgcttgctgtcaaacttctgagttgccgctgatgtgacactgtgacaataaattcaaaccggttatagcggtctcctccggtaccggttctgccacctccaatagagctcagtaggagtcagaacctctgcggtggctgtcagtgactcatccgcgtttcgtaagttgtgcgcgtgcacatttcgcccgttcccgctcatcttgcagcaggcgaaattttcatcacgcggtaggacgcaaaaaaaaaataattaatcgtacaagaatcttggaaaaaaaattgaaaaattttgtataaaagggatgacctaacttgactcaatggcttttacacccagtattttccctttccttgtttgttacaattatagaagcaagacaaaaacatatagacaacctattcctaggagttatatttttttaccctaccagcaatataagtaaaaaataaaacatgttgagaactcaagccgccagattgatctgcaactcccgtgtcatcactgctaagagaacctttgctttggccacccgtgctgctgcttacagcagaccagctgcccgtttcgttaagccaatgatcactacccgtggtttgaagcaaatcaacttcggtggtactgttgaaaccgtctacgaaagagctgactggccaagagaaaagttgttggactacttcaagaacgacacttttgctttgatcggttacggttcccaaggttacggtcaaggtttgaacttgagagacaacggtttgaacgttatcattggtgtccgtaaagatggtgcttcttggaaggctgccatcgaagacggttgggttccaggcaagaacttgttcactgttgaagatgctatcaagagaggttgttacgttatgaacttgttgtccgatgccgctcaatcagaaacctggcctgctatcaagccattgttgaccaagggtaagactttgtacttctcccacggtttctccccagtcttcaaggacttgactcacgttgaaccaccaaaggacttagatgttatcttggttgctccaaagggttccggtagaactgtcagatctttgttcaaggaaggtcgtggtattaactcttcttacgccgtctggaacgatgtcaccggtaaggctcacgaaaaggcccaagctttggccgttgccattggttccggttacgtttaccaaaccactttcgaaagagaagtcaactctgacttgtacggtgaaagaggttgtttaatgggtggtatccacggtatgttcttggctcaatacgacgtcttgagagaaaacggtcactccccatctgaagctttcaacgaaaccgtcgaagaagctacccaatctctatacccattgatcggtaagtacggtatggattacatgtacgatgcttgttccaccaccgccagaagaggtgctttggactggtacccaatcttcaagaatgctttgaagcctgttttccaagacttgtacgaatctaccaagaacggtaccgaaaccaagagatctttggaattcaactctcaacctgactacagagaaaagctagaaaaggaattagacaccatcagaaacatggaaatctggaaggttggtaaggaagtcagaaagttgagaccagaaaaccaataaagaggaaaataatatcaagtgctggaaactttttctcttggaatttttgcaacatcaagtcatagtcaattgaattgacccaatttcacatttaagattttttattttttcatccgacatacatctgtacactaggaagccctgtttttctgaagcagcttcaaatatatatattttttacatatttattatgattcaatgaacaatctaattaaatcgaaaacaagaaccgaaacgcgaataaataatttatttagatggtgacaagtgtataagtcctcatcgggacagctacgatttctctttcggttttggctgagctactggttgctgtgacgcaaactggccaagtgag

SEQ ID NO: 67 - DNA, 20 bp, Artificial
  Primer
  misc_feature (1)..(20): ScILV3_F
tatgttcttattccctcttg

SEQ ID NO: 68 - DNA, 21 bp, Artificial
  Primer
  misc_feature (1)..(21): ScILV3_R
atgtttatccattcaatggac

SEQ ID NO: 69 - DNA, 21 bp, Artificial
  Primer
  misc_feature (1)..(21): ScBAT1_F
atgttgcagagacattccttg

SEQ ID NO: 70 - DNA, 21 bp, Artificial
  Primer
  misc_feature (1)..(21): ScBAT1_R
aggtcaacaatttcaaagagc

SEQ ID NO: 71 - DNA, 25 bp, Artificial
  Primer
  misc_feature (1)..(25): ScBAT2_F
gaccgcactacaccaaagtttaatg

SEQ ID NO: 72 - DNA, 24 bp, Artificial
  Primer
  misc_feature (1)..(24): ScBAT2_R
gataggccagcactagatgacaag

SEQ ID NO: 73 - DNA, 20 bp, Artificial
  Primer
  misc_feature (1)..(20): ScILV6_F
ctaacaagaacggggaatgg

SEQ ID NO: 74 - DNA, 21 bp, Artificial
  Primer
  misc_feature (1)..(21): ScILV6_R
cacttagagaagccaccaagg